European Patent Application EP 4 782 461 A1, published July 29, 2026. Title: A PEPTIDE OR PEPTIDE COCKTAIL AND ITS USE IN THE PREVENTION AND/OR TREATMENT OF AN ORAL INFLAMMATORY DISEASE INDUCED BY ORAL PATHOGENIC BACTERIA OR ANY SYSTEMIC DISEASE WHICH IS NEGATIVELY AFFECTED BY SAID PATHOGENIC BACTERIA. Applicant: Dentaid, S.L. Application EP. The sequence listing filed with the application follows.

SEQUENCE LISTING (12 sequences)

SEQ ID NO: 1 - protein, 18 aa, synthetic construct
  VARIANT 6: note = M, K, G, L, F, I, or T
  VARIANT 9: note = F, W, I, Y, L, or V
  VARIANT 15: note = M, V, S, K, L, I, or Q
KRWKWXKYXHRYFIXHRR

SEQ ID NO: 2 - protein, 18 aa, synthetic construct
KRWKWKKYIHRYFIVHRR

SEQ ID NO: 3 - protein, 18 aa, synthetic construct
KRWKWGKYWHRYFIVHRR

SEQ ID NO: 4 - protein, 18 aa, synthetic construct
KRWKWTKYVHRYFIQHRR

SEQ ID NO: 5 - protein, 18 aa, synthetic construct
KRWKWMKYFHRYFIMHRR

SEQ ID NO: 6 - protein, 18 aa, synthetic construct
KRWKWFKYYHRYFIKHRR

SEQ ID NO: 7 - protein, 18 aa, synthetic construct
KRWKWIKYLHRYFILHRR

SEQ ID NO: 8 - protein, 18 aa, synthetic construct
KRWKWLKYIHRYFISHRR

SEQ ID NO: 9 - protein, 18 aa, synthetic construct
KRWKWIKYYHRYFIIHRR

SEQ ID NO: 10 - protein, 18 aa, synthetic construct
EDQRRDCRREDYCEWARE

SEQ ID NO: 11 - protein, 18 aa, synthetic construct
IYDKKECRKNDDPIEARD

SEQ ID NO: 12 - protein, 18 aa, synthetic construct
KMLKKARRRIECLFYDRE